European Patent Specification EP 3 117 832 B1, published September 27, 2023. Title: Treatment of Microbial Infections. Applicant: The Provost, Fellows, Foundation Scholars, & the other members of Board, of the College of the Holy and Undivided Trinity Of Queen Elizabeth Near Dublin. The sequence listing filed with the application follows.

SEQUENCE LISTING (14 sequences)

SEQ ID NO: 1 - protein, 933 aa, Artificial
  recombinant ClfA (wild type) full length protein sequence
MNMKKKEKHAIRKKSIGVASVLVGTLIGFGLLSSKEADASENSVTQSDSASNESKSNDSSSVSAAPKTDDTNVSDTKTSSNTNNGETSVAQNPAQQETTQSSSTNATTEETPVTGEATTTTTNQANTPATTQSSNTNAEELVNQTSNETTFNDTNTVSSVNSPQNSTNAENVSTTQDTSTEATPSNNESAPQSTDASNKDVVNQAVNTSAPRMRAFSLAAVAADAPAAGTDITNQLTNVTVGIDSGTTVYPHQAGYVKLNYGFSVPNSAVKGDTFKITVPKELNLNGVTSTAKVPPIMAGDQVLANGVIDSDGNVIYTFTDYVNTKDDVKATLTMPAYIDPENVKKTGNVTLATGIGSTTANKTVLVDYEKYGKFYNLSIKGTIDQIDKTNNTYRQTIYVNPSGDNVIAPVLTGNLKPNTDSNALIDQQNTSIKVYKVDNAADLSESYFVNPENFEDVTNSVNITFPNPNQYKVEFNTPDDQITTPYIVVVNGHIDPNSKGDLALRSTLYGYNSNIIWRSMSWDNEVAFNNGSGSGDGIDKPVVPEQPDEPGEIEPIPEDSDSDPGSDSGSDSNSDSGSDSGSDSTSDSGSDSASDSDSASDSDSASDSDSASDSDSASDSDSDNDSDSDSDSDSDSDSDSDSDSDSDSDSDSDSDSDSDSDSDSDSDSDSDSDSDSDSDSDSDSDSDSDSDSDSDSDSDSDSDSDSDSDSDSDSDSDSDSDSDSDSDSDSDSDSDSDSDSDSDSDSDSDSDSDSDSDSDSDSDSDSASDSDSDSDSDSDSDSDSDSDSDSDSDSDSDSDSDSDSDSESDSDSESDSDSDSDSDSDSDSDSDSDSDSASDSDSGSDSDSSSDSDSESDSNSDSESGSNNNVVPPNSPKNGTNASNKNEAKDSKEPLPDTGSEDEANTSLIWGLLASIGSLLLFRRKKENKDKK

SEQ ID NO: 2 - DNA, 1560 bp, Artificial
  recombinant ClfA A domain (wild type) Regions N1 N2 N3
  CDS (1)..(1560)
agtgaaaatagtgttacgcaatctgatagcgcaagtaacgaaagcaaaagtaatgattcaagtagcgttagtgctgcacctaaaacagacgacacaaacgtgagtgatactaaaacatcgtcaaacactaataatggcgaaacgagtgtggcgcaaaatccagcacaacaggaaacgacacaatcatcatcaacaaatgcaactacggaagaaacgccggtaactggtgaagctactactacgacaacgaatcaagctaatacaccggcaacaactcaatcaagcaatacaaatgcggaggaattagtgaatcaaacaagtaatgaaacgacttttaatgatactaatacagtatcatctgtaaattcacctcaaaattctacaaatgcggaaaatgtttcaacaacgcaagatacttcaactgaagcaacaccttcaaacaatgaatcagctccacagagtacagatgcaagtaataaagatgtagttaatcaagcggttaatacaagtgcgcctagaatgagagcatttagtttagcggcagtagctgcagatgcaccggcagctggcacagatattacgaatcagttgacgaatgtgacagttggtattgactctggtacgactgtgtatccgcaccaagcaggttatgtcaaactgaattatggtttttcagtgcctaattctgctgttaaaggtgacacattcaaaataactgtacctaaagaattaaacttaaatggtgtaacttcaactgctaaagtgccaccaattatggctggagatcaagtattggcaaatggtgtaatcgatagtgatggtaatgttatttatacatttacagactatgtaaatactaaagatgatgtaaaagcaactttgaccatgcccgcttatattgaccctgaaaatgttaaaaagacaggtaatgtgacattggctactggcataggtagtacaacagcaaacaaaacagtattagtagattatgaaaaatatggtaagttttataacttatctattaaaggtacaattgaccaaatcgataaaacaaataatacgtatcgtcagacaatttatgtcaatccaagtggagataacgttattgcgccggttttaacaggtaatttaaaaccaaatacggatagtaatgcattaatagatcagcaaaatacaagtattaaagtatataaagtagataatgcagctgatttatctgaaagttactttgtgaatccagaaaactttgaggatgtcactaatagtgtgaatattacattcccaaatccaaatcaatataaagtagagtttaatacgcctgatgatcaaattacaacaccgtatatagtagttgttaatggtcatattgatccgaatagcaaaggtgatttagctttacgttcaactttatatgggtataactcgaatataatttggcgctctatgtcatgggacaacgaagtagcatttaataacggatcaggttctggtgacggtatcgataaaccagttgttcctgaacaacctgatgagcctggtgaaattgaaccaattccagag

SEQ ID NO: 3 - protein, 520 aa, Artificial
  Synthetic Construct
SENSVTQSDSASNESKSNDSSSVSAAPKTDDTNVSDTKTSSNTNNGETSVAQNPAQQETTQSSSTNATTEETPVTGEATTTTTNQANTPATTQSSNTNAEELVNQTSNETTFNDTNTVSSVNSPQNSTNAENVSTTQDTSTEATPSNNESAPQSTDASNKDVVNQAVNTSAPRMRAFSLAAVAADAPAAGTDITNQLTNVTVGIDSGTTVYPHQAGYVKLNYGFSVPNSAVKGDTFKITVPKELNLNGVTSTAKVPPIMAGDQVLANGVIDSDGNVIYTFTDYVNTKDDVKATLTMPAYIDPENVKKTGNVTLATGIGSTTANKTVLVDYEKYGKFYNLSIKGTIDQIDKTNNTYRQTIYVNPSGDNVIAPVLTGNLKPNTDSNALIDQQNTSIKVYKVDNAADLSESYFVNPENFEDVTNSVNITFPNPNQYKVEFNTPDDQITTPYIVVVNGHIDPNSKGDLALRSTLYGYNSNIIWRSMSWDNEVAFNNGSGSGDGIDKPVVPEQPDEPGEIEPIPE

SEQ ID NO: 4 - protein, 520 aa, Artificial
  ClfA A domain Regions N1 N2 N3 with alterations (ClfA P336S Y338A)
SENSVTQSDSASNESKSNDSSSVSAAPKTDDTNVSDTKTSSNTNNGETSVAQNPAQQETTQSSSTNATTEETPVTGEATTTTTNQANTPATTQSSNTNAEELVNQTSNETTFNDTNTVSSVNSPQNSTNAENVSTTQDTSTEATPSNNESAPQSTDASNKDVVNQAVNTSAPRMRAFSLAAVAADAPAAGTDITNQLTNVTVGIDSGTTVYPHQAGYVKLNYGFSVPNSAVKGDTFKITVPKELNLNGVTSTAKVPPIMAGDQVLANGVIDSDGNVIYTFTDYVNTKDDVKATLTMSAAIDPENVKKTGNVTLATGIGSTTANKTVLVDYEKYGKFYNLSIKGTIDQIDKTNNTYRQTIYVNPSGDNVIAPVLTGNLKPNTDSNALIDQQNTSIKVYKVDNAADLSESYFVNPENFEDVTNSVNITFPNPNQYKVEFNTPDDQITTPYIVVVNGHIDPNSKGDLALRSTLYGYNSNIIWRSMSWDNEVAFNNGSGSGDGIDKPVVPEQPDEPGEIEPIPE

SEQ ID NO: 5 - protein, 520 aa, Artificial
  ClfA A domain Regions N1 N2 N3 with alterations (ClfA P336A Y338S)
SENSVTQSDSASNESKSNDSSSVSAAPKTDDTNVSDTKTSSNTNNGETSVAQNPAQQETTQSSSTNATTEETPVTGEATTTTTNQANTPATTQSSNTNAEELVNQTSNETTFNDTNTVSSVNSPQNSTNAENVSTTQDTSTEATPSNNESAPQSTDASNKDVVNQAVNTSAPRMRAFSLAAVAADAPAAGTDITNQLTNVTVGIDSGTTVYPHQAGYVKLNYGFSVPNSAVKGDTFKITVPKELNLNGVTSTAKVPPIMAGDQVLANGVIDSDGNVIYTFTDYVNTKDDVKATLTMAASIDPENVKKTGNVTLATGIGSTTANKTVLVDYEKYGKFYNLSIKGTIDQIDKTNNTYRQTIYVNPSGDNVIAPVLTGNLKPNTDSNALIDQQNTSIKVYKVDNAADLSESYFVNPENFEDVTNSVNITFPNPNQYKVEFNTPDDQITTPYIVVVNGHIDPNSKGDLALRSTLYGYNSNIIWRSMSWDNEVAFNNGSGSGDGIDKPVVPEQPDEPGEIEPIPE

SEQ ID NO: 6 - protein, 530 aa, ARTIFICIAL
  wt rClfA A region with additional N and C terminal residues
HHHHHHGSSENSVTQSDSASNESKSNDSSSVSAAPKTDDTNVSDTKTSSNTNNGETSVAQNPAQQETTQSSSTNATTEETPVTGEATTTTTNQANTPATTQSSNTNAEELVNQTSNETTFNDTNTVSSVNSPQNSTNAENVSTTQDTSTEATPSNNESAPQSTDASNKDVVNQAVNTSAPRMRAFSLAAVAADAPAAGTDITNQLTNVTVGIDSGTTVYPHQAGYVKLNYGFSVPNSAVKGDTFKITVPKELNLNGVTSTAKVPPIMAGDQVLANGVIDSDGNVIYTFTDYVNTKDDVKATLTMPAYIDPENVKKTGNVTLATGIGSTTANKTVLVDYEKYGKFYNLSIKGTIDQIDKTNNTYRQTIYVNPSGDNVIAPVLTGNLKPNTDSNALIDQQNTSIKVYKVDNAADLSESYFVNPENFEDVTNSVNITFPNPNQYKVEFNTPDDQITTPYIVVVNGHIDPNSKGDLALRSTLYGYNSNIIWRSMSWDNEVAFNNGSGSGDGIDKPVVPEQPDEPGEIEPIPEKL

SEQ ID NO: 7 - protein, 530 aa, ARTIFICIAL
  wt rClfAPYI A region with additional N and C terminal residues
HHHHHHGSSENSVTQSDSASNESKSNDSSSVSAAPKTDDTNVSDTKTSSNTNNGETSVAQNPAQQETTQSSSTNATTEETPVTGEATTTTTNQANTPATTQSSNTNAEELVNQTSNETTFNDTNTVSSVNSPQNSTNAENVSTTQDTSTEATPSNNESAPQSTDASNKDVVNQAVNTSAPRMRAFSLAAVAADAPAAGTDITNQLTNVTVGIDSGTTVYPHQAGYVKLNYGFSVPNSAVKGDTFKITVPKELNLNGVTSTAKVPPIMAGDQVLANGVIDSDGNVIYTFTDYVNTKDDVKATLTMSAAIDPENVKKTGNVTLATGIGSTTANKTVLVDYEKYGKFYNLSIKGTIDQIDKTNNTYRQTIYVNPSGDNVIAPVLTGNLKPNTDSNALIDQQNTSIKVYKVDNAADLSESYFVNPENFEDVTNSVNITFPNPNQYKVEFNTPDDQITTPYIVVVNGHIDPNSKGDLALRSTLYGYNSNIIWRSMSWDNEVAFNNGSGSGDGIDKPVVPEQPDEPGEIEPIPEKL

SEQ ID NO: 8 - protein, 530 aa, ARTIFICIAL
  wt rClfAPYII A region with additional N and C terminal residues
HHHHHHGSSENSVTQSDSASNESKSNDSSSVSAAPKTDDTNVSDTKTSSNTNNGETSVAQNPAQQETTQSSSTNATTEETPVTGEATTTTTNQANTPATTQSSNTNAEELVNQTSNETTFNDTNTVSSVNSPQNSTNAENVSTTQDTSTEATPSNNESAPQSTDASNKDVVNQAVNTSAPRMRAFSLAAVAADAPAAGTDITNQLTNVTVGIDSGTTVYPHQAGYVKLNYGFSVPNSAVKGDTFKITVPKELNLNGVTSTAKVPPIMAGDQVLANGVIDSDGNVIYTFTDYVNTKDDVKATLTMAASIDPENVKKTGNVTLATGIGSTTANKTVLVDYEKYGKFYNLSIKGTIDQIDKTNNTYRQTIYVNPSGDNVIAPVLTGNLKPNTDSNALIDQQNTSIKVYKVDNAADLSESYFVNPENFEDVTNSVNITFPNPNQYKVEFNTPDDQITTPYIVVVNGHIDPNSKGDLALRSTLYGYNSNIIWRSMSWDNEVAFNNGSGSGDGIDKPVVPEQPDEPGEIEPIPEKL

SEQ ID NO: 9 - protein, 339 aa, ARTIFICIAL
  rClfA residues 221-559
VAADAPAAGTDITNQLTNVTVGIDSGTTVYPHQAGYVKLNYGFSVPNSAVKGDTFKITVPKELNLNGVTSTAKVPPIMAGDQVLANGVIDSDGNVIYTFTDYVNTKDDVKATLTMPAYIDPENVKKTGNVTLATGIGSTTANKTVLVDYEKYGKFYNLSIKGTIDQIDKTNNTYRQTIYVNPSGDNVIAPVLTGNLKPNTDSNALIDQQNTSIKVYKVDNAADLSESYFVNPENFEDVTNSVNITFPNPNQYKVEFNTPDDQITTPYIVVVNGHIDPNSKGDLALRSTLYGYNSNIIWRSMSWDNEVAFNNGSGSGDGIDKPVVPEQPDEPGEIEPIPE

SEQ ID NO: 10 - protein, 349 aa, ARTIFICIAL
  rClfA residues 221 to 559 with additional N and C terminal residues
HHHHHHGSVAADAPAAGTDITNQLTNVTVGIDSGTTVYPHQAGYVKLNYGFSVPNSAVKGDTFKITVPKELNLNGVTSTAKVPPIMAGDQVLANGVIDSDGNVIYTFTDYVNTKDDVKATLTMPAYIDPENVKKTGNVTLATGIGSTTANKTVLVDYEKYGKFYNLSIKGTIDQIDKTNNTYRQTIYVNPSGDNVIAPVLTGNLKPNTDSNALIDQQNTSIKVYKVDNAADLSESYFVNPENFEDVTNSVNITFPNPNQYKVEFNTPDDQITTPYIVVVNGHIDPNSKGDLALRSTLYGYNSNIIWRSMSWDNEVAFNNGSGSGDGIDKPVVPEQPDEPGEIEPIPEKL

SEQ ID NO: 11 - protein, 339 aa, ARTIFICIAL
  rClfA PY 221 to 559
VAADAPAAGTDITNQLTNVTVGIDSGTTVYPHQAGYVKLNYGFSVPNSAVKGDTFKITVPKELNLNGVTSTAKVPPIMAGDQVLANGVIDSDGNVIYTFTDYVNTKDDVKATLTMSAAIDPENVKKTGNVTLATGIGSTTANKTVLVDYEKYGKFYNLSIKGTIDQIDKTNNTYRQTIYVNPSGDNVIAPVLTGNLKPNTDSNALIDQQNTSIKVYKVDNAADLSESYFVNPENFEDVTNSVNITFPNPNQYKVEFNTPDDQITTPYIVVVNGHIDPNSKGDLALRSTLYGYNSNIIWRSMSWDNEVAFNNGSGSGDGIDKPVVPEQPDEPGEIEPIPE

SEQ ID NO: 12 - protein, 349 aa, ARTIFICIAL
  rClfA PY 221 to 559 with additional N and C terminal residues
HHHHHHGSVAADAPAAGTDITNQLTNVTVGIDSGTTVYPHQAGYVKLNYGFSVPNSAVKGDTFKITVPKELNLNGVTSTAKVPPIMAGDQVLANGVIDSDGNVIYTFTDYVNTKDDVKATLTMSAAIDPENVKKTGNVTLATGIGSTTANKTVLVDYEKYGKFYNLSIKGTIDQIDKTNNTYRQTIYVNPSGDNVIAPVLTGNLKPNTDSNALIDQQNTSIKVYKVDNAADLSESYFVNPENFEDVTNSVNITFPNPNQYKVEFNTPDDQITTPYIVVVNGHIDPNSKGDLALRSTLYGYNSNIIWRSMSWDNEVAFNNGSGSGDGIDKPVVPEQPDEPGEIEPIPEKL

SEQ ID NO: 13 - protein, 321 aa, ARTIFICIAL
  rClfA residues 221 to 531 with additional N and C terminal residues (delta latch truncate)
HHHHHHGSVAADAPAAGTDITNQLTNVTVGIDSGTTVYPHQAGYVKLNYGFSVPNSAVKGDTFKITVPKELNLNGVTSTAKVPPIMAGDQVLANGVIDSDGNVIYTFTDYVNTKDDVKATLTMPAYIDPENVKKTGNVTLATGIGSTTANKTVLVDYEKYGKFYNLSIKGTIDQIDKTNNTYRQTIYVNPSGDNVIAPVLTGNLKPNTDSNALIDQQNTSIKVYKVDNAADLSESYFVNPENFEDVTNSVNITFPNPNQYKVEFNTPDDQITTPYIVVVNGHIDPNSKGDLALRSTLYGYNSNIIWRSMSWDNEVAFNNRS

SEQ ID NO: 14 - protein, 311 aa, ARTIFICIAL
  rClfA residues 221 to 531 (delta latch truncate)
VAADAPAAGTDITNQLTNVTVGIDSGTTVYPHQAGYVKLNYGFSVPNSAVKGDTFKITVPKELNLNGVTSTAKVPPIMAGDQVLANGVIDSDGNVIYTFTDYVNTKDDVKATLTMPAYIDPENVKKTGNVTLATGIGSTTANKTVLVDYEKYGKFYNLSIKGTIDQIDKTNNTYRQTIYVNPSGDNVIAPVLTGNLKPNTDSNALIDQQNTSIKVYKVDNAADLSESYFVNPENFEDVTNSVNITFPNPNQYKVEFNTPDDQITTPYIVVVNGHIDPNSKGDLALRSTLYGYNSNIIWRSMSWDNEVAFNN